European Patent Specification EP 4 333 867 B1, published December 18, 2024. Title: Covid-19 blocking peptide. Applicant: QuantBioRes A/S. The sequence listing filed with the application follows.

SEQUENCE LISTING (6 sequences)

SEQ ID NO: 1 - protein, 18 aa, Artificial Sequence
  synthetic peptide
  MISC_FEATURE (1)..(18): CovA
HRWKQWWWAQCPYDKLDM

SEQ ID NO: 2 - protein, 18 aa, Artificial Sequence
  synthetic peptide
  MISC_FEATURE (1)..(18): CovB
LWDKERTNWDAERRGYDY

SEQ ID NO: 3 - protein, 18 aa, Artificial Sequence
  synthetic peptide
  MISC_FEATURE (1)..(18): CovC
QDEWDHKDAPDWGRCLTR

SEQ ID NO: 4 - protein, 18 aa, Artificial Sequence
  synthetic peptide
  MISC_FEATURE (1)..(18): CovD
RHWFWWQQCWARMVTDLY

SEQ ID NO: 5 - protein, 18 aa, Artificial Sequence
  synthetic peptide
  MISC_FEATURE (1)..(18): CovE
DWNTDPKDQICDPHDQLQ

SEQ ID NO: 6 - protein, 18 aa, Artificial Sequence
  synthetic peptide
  MISC_FEATURE (1)..(18): CovF
YEDQNRTLCRVWDPKDKP